European Patent Application EP 4 130 268 A1, published February 8, 2023. Title: CpG ODN Having Immunoregulatory Function and Use Thereof. Applicant: Parr Biotechnology (Hebei) Co., Ltd. The sequence listing filed with the application follows.

SEQUENCE LISTING (8 sequences)

SEQ ID NO: 1 - DNA, 26 bp, artificial sequence
  artificially synthesized nucleotide sequence
tcgcgacgttcgcgggacgttcccta

SEQ ID NO: 2 - DNA, 26 bp, artificial sequence
  artificially synthesized nucleotide sequence
tcgcgacgttcgcgcgacgttcgcta

SEQ ID NO: 3 - DNA, 24 bp, artificial sequence
  artificially synthesized nucleotide sequence
tcgcgacgttcgccgacgttcgta

SEQ ID NO: 4 - DNA, 23 bp, artificial sequence
  artificially synthesized nucleotide sequence
tggacgttcgtcgttcgtccttc

SEQ ID NO: 5 - DNA, 23 bp, artificial sequence
  artificially synthesized nucleotide sequence
tcgtcgttcgtcgttcgacgttc

SEQ ID NO: 6 - DNA, 23 bp, artificial sequence
  artificially synthesized nucleotide sequence
tcgaggttcgtcgttcctcgttc

SEQ ID NO: 7 - DNA, 22 bp, artificial sequence
  artificially synthesized nucleotide sequence
tgactgtgaacgttcgagatga

SEQ ID NO: 8 - DNA, 29 bp, artificial sequence
  artificially synthesized nucleotide sequence
tggccaagcttgggccccttgcaagggcc